European Patent Application EP 4 442 279 A1, published October 9, 2024. Title: Immunostimulatory Composition. Applicant: Reiko Shinkura. Application EP 22901178.8, filed November 24, 2022. The sequence listing filed with the application follows.

SEQUENCE LISTING (10 sequences)

SEQ ID NO: 1 - DNA, 20 bp, synthetic construct
  source 1..20: mol_type = other DNA
  misc_difference 1: note = s denotes c or g
  misc_difference 13: note = s denotes c or g
  misc_difference 16: note = s denotes c or g
  misc_difference 3: note = r denotes a or g
  misc_difference 6: note = n denotes a, g, c or t
  misc_difference 7: note = m denotes a or c
sargtnmagctgsagsagtc

SEQ ID NO: 2 - DNA, 23 bp, synthetic construct
  source 1..23: mol_type = other DNA
  misc_difference 1: note = s denotes c or g
  misc_difference 3: note = r denotes a or g
  misc_difference 6: note = n denotes a, g, c or t
  misc_difference 7: note = m denotes a or c
  misc_difference 13: note = s denotes c or g
  misc_difference 16: note = s denotes c or g
  misc_difference 21: note = w denotes a or t
sargtnmagctgsagsagtcwgg

SEQ ID NO: 3 - DNA, 22 bp, synthetic construct
  source 1..22: mol_type = other DNA
  misc_difference 17: note = w denotes a or t
  misc_difference 20: note = s denotes c or g
caggttactctgaaagwgtstg

SEQ ID NO: 4 - DNA, 20 bp, synthetic construct
  source 1..20: mol_type = other DNA
  misc_difference 9: note = r denotes a or g
  misc_difference 18: note = r denotes a or g
gaggtccarctgcaacartc

SEQ ID NO: 5 - DNA, 20 bp, synthetic construct
  source 1..20: mol_type = other DNA
  misc_difference 18: note = r denotes a or g
caggtccaactvcagcarcc

SEQ ID NO: 6 - DNA, 20 bp, synthetic construct
  source 1..20: mol_type = other DNA
  misc_difference 9: note = s denotes c or g
  misc_difference 10: note = s denotes c or g
gaggtgaasstggtggaatc

SEQ ID NO: 7 - DNA, 20 bp, synthetic construct
  source 1..20: mol_type = other DNA
gatgtgaacttggaagtgtc

SEQ ID NO: 8 - DNA, 30 bp, synthetic construct
  source 1..30: mol_type = other DNA
gactagtcctctccagtttcggctgaatcc

SEQ ID NO: 9 - DNA, 18 bp, synthetic construct
  source 1..18: mol_type = other DNA
caggtggtgttttgctca

SEQ ID NO: 10 - DNA, 18 bp, synthetic construct
  source 1..18: mol_type = other DNA
tatgctatggactactgg